European Patent Application EP 4 230 640 A1, published August 23, 2023. Title: GLP-1/GIP dual agonist, a long acting conjugate thereof, and a pharmaceutical composition comprising the same. Applicant: HANMI PHARM. CO., LTD. The sequence listing filed with the application follows.

SEQUENCE LISTING (64 sequences)

SEQ ID NO: 1 - protein, 40 aa, Artificial
  GLP-1/GIP dual agonist
  MISC_FEATURE (2)..(2): Xaa is aminoisobutyric acid (Aib)
  MISC_FEATURE (12)..(16): amino acids at positions 12 and 16 form a ring
YXEGTFTSDYSEYMEKEAVREFIAWLVKGGPSSGAPPPSC

SEQ ID NO: 2 - protein, 40 aa, Artificial
  GLP-1/GIP dual agonist
  MISC_FEATURE (2)..(2): Xaa is aminoisobutyric acid (Aib)
  MISC_FEATURE (16)..(20): amino acids at positions 16 and 20 form a ring
YXEGTFTSDYSKYLDEIRAKDFVQWLLDHHPSSGQPPPSC

SEQ ID NO: 3 - protein, 40 aa, Artificial
  GLP-1/GIP dual agonist
  MISC_FEATURE (2)..(2): Xaa is aminoisobutyric acid (Aib)
  MISC_FEATURE (16)..(20): amino acids at positions 16 and 20 form a ring
YXEGTFTSDYSKYLDEIAAKDFVQWLLDHHPSSGQPPPSC

SEQ ID NO: 4 - protein, 39 aa, Artificial
  GLP-1/GIP dual agonist
  MISC_FEATURE (2)..(2): Xaa is aminoisobutyric acid (Aib)
  MISC_FEATURE (16)..(20): amino acids at positions 16 and 20 form a ring
YXEGTFTSDYSKYLDEIRAKDFVQWLLDHHPSSGQPPPC

SEQ ID NO: 5 - protein, 40 aa, Artificial
  GLP-1/GIP dual agonist
  MISC_FEATURE (2)..(2): Xaa is aminoisobutyric acid (Aib)
  MISC_FEATURE (16)..(20): amino acids at positions 16 and 20 form a ring
YXEGTFTSDYSKYLDEKAAKDFVQWLLDHHPSSGQPPPSC

SEQ ID NO: 6 - protein, 40 aa, Artificial
  GLP-1/GIP dual agonist
  MISC_FEATURE (2)..(2): Xaa is aminoisobutyric acid (Aib)
  MISC_FEATURE (16)..(20): amino acids at positions 16 and 20 form a ring
YXEGTFTSDYSKYLDEKRAKDFVQWLLDHHPSSGQPPPSC

SEQ ID NO: 7 - protein, 40 aa, Artificial
  GLP-1/GIP dual agonist
  MISC_FEATURE (2)..(2): Xaa is aminoisobutyric acid (Aib)
  MISC_FEATURE (16)..(20): amino acids at positions 16 and 20 form a ring
YXEGTFTSDYSKYLDERAQKDFVQWLLDHHPSSGQPPPSC

SEQ ID NO: 8 - protein, 40 aa, Artificial
  GLP-1/GIP dual agonist
  MISC_FEATURE (2)..(2): Xaa is aminoisobutyric acid (Aib)
  MISC_FEATURE (16)..(20): amino acids at positions 16 and 20 form a ring
YXEGTFTSDYSKYLDERASKDFVQWLLDHHPSSGQPPPSC

SEQ ID NO: 9 - protein, 40 aa, Artificial
  GLP-1/GIP dual agonist
  MISC_FEATURE (2)..(2): Xaa is aminoisobutyric acid (Aib)
  MISC_FEATURE (16)..(20): amino acids at positions 16 and 20 form a ring
YXEGTFTSDYSRYLDERAAKDFVQWLLDHHPSSGQPPPSK

SEQ ID NO: 10 - protein, 40 aa, Artificial
  GLP-1/GIP dual agonist
  MISC_FEATURE (2)..(2): Xaa is aminoisobutyric acid (Aib)
  MISC_FEATURE (16)..(20): amino acids at positions 16 and 20 form a ring
YXEGTFTSDYSRYLDERAQKDFVQWLLDHHPSSGQPPPSK

SEQ ID NO: 11 - protein, 40 aa, Artificial
  GLP-1/GIP dual agonist
  MISC_FEATURE (2)..(2): Xaa is aminoisobutyric acid (Aib)
  MISC_FEATURE (16)..(20): amino acids at positions 16 and 20 form a ring
YXEGTFTSDYSRYLDERASKDFVQWLLDHHPSSGQPPPSK

SEQ ID NO: 12 - protein, 40 aa, Artificial
  GLP-1/GIP dual agonist
  MISC_FEATURE (2)..(2): Xaa is aminoisobutyric acid (Aib)
  MISC_FEATURE (12)..(16): amino acids at positions 12 and 16 form a ring
YXEGTFTSDYSEYMEKEAVREFIAWLVRGGPSSGAPPPSK

SEQ ID NO: 13 - protein, 40 aa, Artificial
  GLP-1/GIP dual agonist
  MISC_FEATURE (2)..(2): Xaa is aminoisobutyric acid (Aib)
  MISC_FEATURE (12)..(16): amino acids at positions 12 and 16 form a ring
YXEGTFTSDYSEYMEKEAVREFISWLVRGGPSSGAPPPSK

SEQ ID NO: 14 - protein, 40 aa, Artificial
  GLP-1/GIP dual agonist
  MISC_FEATURE (2)..(2): Xaa is aminoisobutyric acid (Aib)
  MISC_FEATURE (20)..(20): X is aminoisobutyric acid (Aib)
HXEGTFTSDYSKYLDKKRQXEFVQWLLNGGPSSGAPPPSC

SEQ ID NO: 15 - protein, 41 aa, Artificial
  GLP-1/GIP dual agonist
  MISC_FEATURE (2)..(2): Xaa is aminoisobutyric acid (Aib)
  MISC_FEATURE (16)..(20): amino acids at positions 16 and 20 form a ring
YXEGTFTSDYSIYLDERACKDFVQWLLDHHPSSGQPPPSYK

SEQ ID NO: 16 - protein, 40 aa, Artificial
  GLP-1/GIP dual agonist
  MISC_FEATURE (2)..(2): Xaa is aminoisobutyric acid (Aib)
  MISC_FEATURE (13)..(13): X is aminoisobutyric acid (Aib)
YXEGTFTSDYSIXLDKIAQRAFVQWLIAGGPSSGAPPPSK

SEQ ID NO: 17 - protein, 40 aa, Artificial
  GLP-1/GIP dual agonist
  MISC_FEATURE (2)..(2): Xaa is aminoisobutyric acid (Aib)
YXEGTFTSDYSIQLDKIAQKAFVQWLIAGGPSSGAPPPSC

SEQ ID NO: 18 - protein, 40 aa, Artificial
  GLP-1/GIP dual agonist
  MISC_FEATURE (2)..(2): Xaa is aminoisobutyric acid (Aib)
YXEGTFTSDYSIQLDKIAQRAFVQWLIAGGPSSGAPPPSK

SEQ ID NO: 19 - protein, 40 aa, Artificial
  GLP-1/GIP dual agonist
  MISC_FEATURE (2)..(2): Xaa is aminoisobutyric acid (Aib)
  MISC_FEATURE (20)..(20): Xaa is aminoisobutyric acid (Aib)
YXEGTFTSDYSIYLDKQAAXAFVQWLIAGGPSSGAPPPSC

SEQ ID NO: 20 - protein, 40 aa, Artificial
  GLP-1/GIP dual agonist
  MISC_FEATURE (2)..(2): Xaa is aminoisobutyric acid (Aib)
  MISC_FEATURE (13)..(13): Xaa is aminoisobutyric acid (Aib)
  MISC_FEATURE (20)..(20): Xaa is aminoisobutyric acid (Aib)
YXEGTFTSDYSIXLDKQAAXAFVQWLIAGGPSSGAPPPSC

SEQ ID NO: 21 - protein, 40 aa, Artificial
  GLP-1/GIP dual agonist
  MISC_FEATURE (2)..(2): Xaa is aminoisobutyric acid (Aib)
  MISC_FEATURE (13)..(13): Xaa is aminoisobutyric acid (Aib)
YXEGTFTSDYSIXLDKIAAKAFVQWLIAGGPSSGAPPPSC

SEQ ID NO: 22 - protein, 40 aa, Artificial
  GLP-1/GIP dual agonist
  MISC_FEATURE (2)..(2): Xaa is aminoisobutyric acid (Aib)
  MISC_FEATURE (16)..(20): amino acids at positions 16 and 20 form a ring
YXEGTFTSDYSKYLDEKAAKEFVQWLLDQHPSSGQPPPSC

SEQ ID NO: 23 - protein, 40 aa, Artificial
  GLP-1/GIP dual agonist
  MISC_FEATURE (2)..(2): Xaa is aminoisobutyric acid (Aib)
  MISC_FEATURE (16)..(20): amino acids at positions 16 and 20 form a ring
YXEGTFTSDYSKYLDEQAAKEFVQWLLDQHPSSGAPPPSC

SEQ ID NO: 24 - protein, 40 aa, Artificial
  GLP-1/GIP dual agonist
  MISC_FEATURE (2)..(2): Xaa is aminoisobutyric acid (Aib)
  MISC_FEATURE (16)..(20): amino acids at positions 16 and 20 form a ring
YXEGTFTSDYSKYLDEIAQKDFVQWLLDQHPSSGAPPPSC

SEQ ID NO: 25 - protein, 40 aa, Artificial
  GLP-1/GIP dual agonist
  MISC_FEATURE (2)..(2): Xaa is aminoisobutyric acid (Aib)
  MISC_FEATURE (16)..(20): amino acids at positions 16 and 20 form a ring
YXEGTFTSDYSKYLDEEAVKLFVQWLLDQHPSSGAPPPSC

SEQ ID NO: 26 - protein, 43 aa, Artificial
  GLP-1/GIP dual agonist
  MISC_FEATURE (2)..(2): Xaa is aminoisobutyric acid (Aib)
YXEGTFTSDYSIAMDAIAQQDFVNWLLAQKGKKNDWKHNITQC

SEQ ID NO: 27 - protein, 43 aa, Artificial
  GLP-1/GIP dual agonist
  MISC_FEATURE (2)..(2): Xaa is aminoisobutyric acid (Aib)
YXEGTFTSDYSIAMDAIAQQDFVNWLLAQRGKKSDWKHNITQC

SEQ ID NO: 28 - protein, 40 aa, Artificial
  GLP-1/GIP dual agonist
  MISC_FEATURE (2)..(2): Xaa is aminoisobutyric acid (Aib)
YXEGTFTSDYSIALEKQAQQDFVNWLLAGGPSSGAPPPSC

SEQ ID NO: 29 - protein, 40 aa, Artificial
  GLP-1/GIP dual agonist
  MISC_FEATURE (2)..(2): Xaa is aminoisobutyric acid (Aib)
  MISC_FEATURE (13)..(13): Xaa is aminoisobutyric acid (Aib)
  MISC_FEATURE (20)..(20): Xaa is aminoisobutyric acid (Aib)
  MISC_FEATURE (28)..(28): Xaa is aminoisobutyric acid (Aib)
YXEGTFTSDYSIXLDKQAAXEFVNWLLXGGPSSGAPPPSC

SEQ ID NO: 30 - protein, 40 aa, Artificial
  GLP-1/GIP dual agonist
  MISC_FEATURE (2)..(2): Xaa is aminoisobutyric acid (Aib)
  MISC_FEATURE (13)..(13): Xaa is aminoisobutyric acid (Aib)
  MISC_FEATURE (20)..(20): Xaa is aminoisobutyric acid (Aib)
  MISC_FEATURE (28)..(28): Xaa is aminoisobutyric acid (Aib)
YXEGTFTSDYSIXLDKQAAXEFVNWLLXGHPSSGAPPPSC

SEQ ID NO: 31 - protein, 40 aa, Artificial
  GLP-1/GIP dual agonist
  MISC_FEATURE (1)..(1): Xaa is 3-(4-hydroxyphenyl)propanoic acid (HP)
  MISC_FEATURE (2)..(2): Xaa is aminoisobutyric acid (Aib)
  MISC_FEATURE (13)..(13): Xaa is aminoisobutyric acid (Aib)
XXEGTFTSDYSIXLDKIAQRAFVQWLIAGGPSSGAPPPSK

SEQ ID NO: 32 - protein, 40 aa, Artificial; identical to SEQ ID NO: 31
  GLP-1/GIP dual agonist
  MISC_FEATURE (1)..(1): Xaa is 2-(4-hydroxyphenyl)acetic acid (HA)
  MISC_FEATURE (2)..(2): Xaa is aminoisobutyric acid (Aib)
  MISC_FEATURE (13)..(13): Xaa is aminoisobutyric acid (Aib)

SEQ ID NO: 33 - protein, 41 aa, Artificial
  GLP-1/GIP dual agonist
  MISC_FEATURE (1)..(1): Xaa is 4-imidazoleacetic acid (CA)
  MISC_FEATURE (3)..(3): Xaa is aminoisobutyric acid (Aib)
  MISC_FEATURE (14)..(14): Xaa is aminoisobutyric acid (Aib)
XYXEGTFTSDYSIXLDKIAQRAFVQWLIAGGPSSGAPPPSK

SEQ ID NO: 34 - protein, 40 aa, Artificial
  GLP-1/GIP dual agonist
  MISC_FEATURE (2)..(2): Xaa is aminoisobutyric acid (Aib)
  MISC_FEATURE (13)..(13): Xaa is aminoisobutyric acid (Aib)
YXEGTFTSDYSIXLDKQAARAFVQWLIAGGPSSGAPPPSC

SEQ ID NO: 35 - protein, 40 aa, Artificial
  GLP-1/GIP dual agonist
  MISC_FEATURE (2)..(2): Xaa is aminoisobutyric acid (Aib)
  MISC_FEATURE (13)..(13): Xaa is aminoisobutyric acid (Aib)
  MISC_FEATURE (20)..(20): Xaa is aminoisobutyric acid (Aib)
YXEGTFTSDYSIXLDKQHAXAFVQWLIAGGPSSGAPPPSC

SEQ ID NO: 36 - protein, 40 aa, Artificial
  GLP-1/GIP dual agonist
  MISC_FEATURE (2)..(2): Xaa is aminoisobutyric acid (Aib)
  MISC_FEATURE (13)..(13): Xaa is aminoisobutyric acid (Aib)
YXEGTFTSDYSIXLDKQAQQAFVQWLIAGGPSSGAPPPSC

SEQ ID NO: 37 - protein, 40 aa, Artificial
  GLP-1/GIP dual agonist
  MISC_FEATURE (2)..(2): Xaa is aminoisobutyric acid (Aib)
  MISC_FEATURE (13)..(13): Xaa is aminoisobutyric acid (Aib)
  MISC_FEATURE (20)..(20): Xaa is aminoisobutyric acid (Aib)
  misc_feature (21)..(21): Xaa can be any naturally occurring amino acid
YXEGTFTSDYSIXLDKQAQQXFVQWLIAGGPSSGAPPPSC

SEQ ID NO: 38 - protein, 40 aa, Artificial
  GLP-1/GIP dual agonist
  MISC_FEATURE (2)..(2): Xaa is aminoisobutyric acid (Aib)
  MISC_FEATURE (13)..(13): Xaa is aminoisobutyric acid (Aib)
YXEGTFTSDYSIXLEKQAQQDFVNWLLAGGPSSGAPPPSC

SEQ ID NO: 39 - protein, 40 aa, Artificial
  GLP-1/GIP dual agonist
  MISC_FEATURE (2)..(2): Xaa is aminoisobutyric acid (Aib)
  MISC_FEATURE (20)..(20): Xaa is aminoisobutyric acid (Aib)
YXEGTFTSDYSIALEKQAAXDFVNWLLAGGPSSGAPPPSC

SEQ ID NO: 40 - protein, 40 aa, Artificial
  GLP-1/GIP dual agonist
  MISC_FEATURE (2)..(2): Xaa is aminoisobutyric acid (Aib)
YXEGTFTSDYSIALEKQAQRDFVNWLLAGGPSSGAPPPSC

SEQ ID NO: 41 - protein, 40 aa, Artificial
  GLP-1/GIP dual agonist
  MISC_FEATURE (1)..(1): Xaa is 3-(4-hydroxyphenyl)propanoic acid (HP)
  MISC_FEATURE (2)..(2): Xaa is aminoisobutyric acid (Aib)
  MISC_FEATURE (13)..(13): Xaa is aminoisobutyric acid (Aib)
  MISC_FEATURE (20)..(20): Xaa is aminoisobutyric acid (Aib)
XXEGTFTSDYSIXLDAQAAXAFVQWLIAGGPSSGAPPPSK

SEQ ID NO: 42 - protein, 40 aa, Artificial
  GLP-1/GIP dual agonist
  MISC_FEATURE (1)..(1): Xaa is 3-(4-hydroxyphenyl)propanoic acid (HP)
  MISC_FEATURE (2)..(2): Xaa is aminoisobutyric acid (Aib)
  MISC_FEATURE (13)..(13): Xaa is aminoisobutyric acid (Aib)
  MISC_FEATURE (16)..(16): Xaa is Norleucine (Nle)
  MISC_FEATURE (20)..(20): Xaa is aminoisobutyric acid (Aib)
XXEGTFTSDYSIXLDXQAAXAFVQWLIAGGPSSGAPPPSK

SEQ ID NO: 43 - protein, 40 aa, Artificial
  GLP-1/GIP dual agonist
  MISC_FEATURE (1)..(1): Xaa is 3-(4-hydroxyphenyl)propanoic acid (HP)
  MISC_FEATURE (2)..(2): Xaa is aminoisobutyric acid (Aib)
XXEGTFISDYSIALEAQAQQDFVNWLLAGGPSSGAPPPSK

SEQ ID NO: 44 - protein, 40 aa, Artificial
  GLP-1/GIP dual agonist
  MISC_FEATURE (1)..(1): Xaa is 3-(4-hydroxyphenyl)propanoic acid (HP)
  MISC_FEATURE (2)..(2): Xaa is aminoisobutyric acid (Aib)
  MISC_FEATURE (16)..(16): Xaa is Norleucine (Nle)
XXEGTFISDYSIALEXQAQQDFVNWLLAGGPSSGAPPPSK

SEQ ID NO: 45 - protein, 12 aa, Homo sapiens
ESKYGPPCPSCP

SEQ ID NO: 46 - protein, 11 aa, Artificial
  Variant of hinge region
ESKYGPPPSCP

SEQ ID NO: 47 - protein, 11 aa, Artificial
  Variant of hinge region
ESKYGPPCPSP

SEQ ID NO: 48 - protein, 10 aa, Artificial
  Variant of hinge region
ESKYGPPCPS

SEQ ID NO: 49 - protein, 10 aa, Artificial
  Variant of hinge region
ESKYGPPCPP

SEQ ID NO: 50 - protein, 8 aa, Artificial
  Variant of hinge region
KYGPPCPS

SEQ ID NO: 51 - protein, 8 aa, Artificial
  Variant of hinge region
ESKYGPPC

SEQ ID NO: 52 - protein, 7 aa, Artificial
  Variant of hinge region
EKYGPPC

SEQ ID NO: 53 - protein, 6 aa, Artificial
  Variant of hinge region
ESPSCP

SEQ ID NO: 54 - protein, 5 aa, Artificial
  Variant of hinge region
EPSCP

SEQ ID NO: 55 - protein, 4 aa, Artificial
  Variant of hinge region
PSCP

SEQ ID NO: 56 - protein, 10 aa, Artificial
  Variant of hinge region
ESKYGPPSCP

SEQ ID NO: 57 - protein, 9 aa, Artificial
  Variant of hinge region
KYGPPPSCP

SEQ ID NO: 58 - protein, 9 aa, Artificial
  Variant of hinge region
ESKYGPSCP

SEQ ID NO: 59 - protein, 8 aa, Artificial
  Variant of hinge region
ESKYGPPC

SEQ ID NO: 60 - protein, 7 aa, Artificial
  Variant of hinge region
KYGPPCP

SEQ ID NO: 61 - protein, 7 aa, Artificial
  Variant of hinge region
ESKPSCP

SEQ ID NO: 62 - protein, 6 aa, Artificial
  Variant of hinge region
ESPSCP

SEQ ID NO: 63 - protein, 4 aa, Artificial
  Variant of hinge region
EPSC

SEQ ID NO: 64 - protein, 3 aa, Artificial
  Variant of hinge region
SCP